European Patent Application EP 4 717 710 A1, published April 1, 2026. Title: A Novel Nanobody Binding to Human Interleukin-4 Receptor and a Formulation for Nasal Spray Comprising the Same. Applicant: Yonsei University Industry Academic Cooperation Foundation. Application KR. The sequence listing filed with the application follows.

SEQUENCE LISTING (23 sequences)

SEQ ID NO: 1 - protein, 16 aa, synthetic construct
DKGREYTLARAKYWYW

SEQ ID NO: 2 - protein, 16 aa, synthetic construct
DKGRRYTLARAKYWYW

SEQ ID NO: 3 - protein, 16 aa, synthetic construct
DKGREYTLARYKYWYW

SEQ ID NO: 4 - protein, 16 aa, synthetic construct
DKGRRYTLARYKYWYW

SEQ ID NO: 5 - protein, 150 aa, synthetic construct
QVQLVESGGGSVQAGGSLRLSCAASGSISSITYLGWFRQAPGKEREGVAALSTSSGTTYYADSVKGRFTVSLDNAKNTVYLQMNSLKPEDTALYYCAAADKGREYTLARAKYWYWGQGTQVTVSAGRAGEQKLISEEDLNSAVDHHHHHH

SEQ ID NO: 6 - protein, 150 aa, synthetic construct
QVQLVESGGGSVQAGGSLRLSCAASGSISSITYLGWFRQAPGKEREGVAALSTSSGTTYYADSVKGRFTVSLDNAKNTVYLQMNSLKPEDTALYYCAAADKGRRYTLARAKYWYWGQGTQVTVSAGRAGEQKLISEEDLNSAVDHHHHHH

SEQ ID NO: 7 - protein, 150 aa, synthetic construct
QVQLVESGGGSVQAGGSLRLSCAASGSISSITYLGWFRQAPGKEREGVAALSTSSGTTYYADSVKGRFTVSLDNAKNTVYLQMNSLKPEDTALYYCAAADKGREYTLARYKYWYWGQGTQVTVSAGRAGEQKLISEEDLNSAVDHHHHHH

SEQ ID NO: 8 - protein, 150 aa, synthetic construct
QVQLVESGGGSVQAGGSLRLSCAASGSISSITYLGWFRQAPGKEREGVAALSTSSGTTYYADSVKGRFTVSLDNAKNTVYLQMNSLKPEDTALYYCAAADKGRRYTLARYKYWYWGQGTQVTVSAGRAGEQKLISEEDLNSAVDHHHHHH

SEQ ID NO: 9 - skipped

SEQ ID NO: 10 - DNA, 21 bp, synthetic construct
  source 1..21: mol_type = other DNA
caagtccagctggtggaatcg

SEQ ID NO: 11 - DNA, 16 bp, synthetic construct
  source 1..16: mol_type = other DNA
gccgctagccgcacag

SEQ ID NO: 12 - DNA, 23 bp, synthetic construct
  source 1..23: mol_type = other DNA
atatatgaagacctctgcgcggc

SEQ ID NO: 13 - DNA, 40 bp, synthetic construct
  source 1..40: mol_type = other DNA
atgcatggtctcagcagtaatacaaagcagtatcttccgg

SEQ ID NO: 14 - DNA, 66 bp, synthetic construct
  source 1..66: mol_type = other DNA
gaagacctctgcgcggcagccggcccgctgtattactggggtcagggcacccaagttaccgtttct

SEQ ID NO: 15 - DNA, 30 bp, synthetic construct
  source 1..30: mol_type = other DNA
cgaaattaatacgactcactatagggagac

SEQ ID NO: 16 - DNA, 33 bp, synthetic construct
  source 1..33: mol_type = other DNA
tatagctcttcaactacccatggatatatctcc

SEQ ID NO: 17 - DNA, 32 bp, synthetic construct
  source 1..32: mol_type = other DNA
tatagctcttctgcaaagctttatatggcctc

SEQ ID NO: 18 - DNA, 45 bp, synthetic construct
  source 1..45: mol_type = other DNA
ccgcacaccagtaaggtgtgcggtttcagttgccgctttctttct

SEQ ID NO: 19 - DNA, 24 bp, synthetic construct
  source 1..24: mol_type = other DNA
cttcagttgccgctttctttcttg

SEQ ID NO: 20 - DNA, 36 bp, synthetic construct
  source 1..36: mol_type = other DNA
atatgctcttctagtcaagtccagctggtggaatcg

SEQ ID NO: 21 - DNA, 37 bp, synthetic construct
  source 1..37: mol_type = other DNA
tatagctcttcatgcagaaacggtaacttgggtgccc

SEQ ID NO: 22 - DNA, 21 bp, synthetic construct
  source 1..21: mol_type = other DNA
gggagaccacaacggtttccc

SEQ ID NO: 23 - DNA, 19 bp, synthetic construct
  source 1..19: mol_type = other DNA
gccgctagccgcacagctc